European Patent Application EP 4 234 713 A2, published August 30, 2023. Title: METHODS OF LOWERING THE ERROR RATE OF MASSIVELY PARALLEL DNA SEQUENCING USING DUPLEX CONSENSUS SEQUENCING. Applicant: University of Washington through its Center for Commercialization. Application EP 13764186.6. The sequence listing filed with the application follows.

SEQUENCE LISTING (9 sequences)

SEQ ID NO: 1 - DNA, 58 bp, synthetic construct
  misc_feature 1..58: note = Synthetic oligonucleotide
  source 1..58: mol_type = other DNA
aatgatacggcgaccaccgagatctacactctttccctacacgacgctcttccgatct

SEQ ID NO: 2 - DNA, 50 bp, synthetic construct
  misc_feature 1..50: note = Synthetic oligonucleotide
  misc_feature 5..16: note = n is a, c, g, or t
  source 1..50: mol_type = other DNA
actgnnnnnnnnnnnnagatcggaagagcacacgtctgaactccagtcac

SEQ ID NO: 3 - DNA, 21 bp, synthetic construct
  misc_feature 1..21: note = Synthetic oligonucleotide
  source 1..21: mol_type = other DNA
aatgatacggcgaccaccgag

SEQ ID NO: 4 - DNA, 23 bp, synthetic construct
  misc_feature 1..23: note = Synthetic oligonucleotide
  source 1..23: mol_type = other DNA
gtgactggagttcagacgtgtgc

SEQ ID NO: 5 - DNA, 53 bp, synthetic construct
  misc_feature 1..53: note = Synthetic oligonucleotide
  misc_feature 25..30: note = position of fixed multiplexing barcode sequence
  misc_feature 25..30: note = n is a, c, g, or t
  source 1..53: mol_type = other DNA
caagcagaagacggcatacgagatnnnnnngtgactggagttcagacgtgtgc

SEQ ID NO: 6-9 - skipped (4 entries)